European Patent Application EP 4 400 591 A1, published July 17, 2024. Title: INDUCIBLE PROMOTER, VECTOR AND HOST CELL BASED THEREON. Applicant: Joint Stock Company «BIOCAD». Application WO PCT/RU2022/050279, filed September 6, 2022. The sequence listing filed with the application follows.

SEQUENCE LISTING (16 sequences)

SEQ ID NO: 1 - DNA, 17 bp, Naturally occurring sequence
  source 1..17: mol_type = genomic DNA
agggttcctggaaggga

SEQ ID NO: 2 - DNA, 17 bp, Naturally occurring sequence
  source 1..17: mol_type = genomic DNA
cagattccgggaatccc

SEQ ID NO: 3 - DNA, 17 bp, Naturally occurring sequence
  source 1..17: mol_type = genomic DNA
atccttctgggaattct

SEQ ID NO: 4 - DNA, 17 bp, Naturally occurring sequence
  source 1..17: mol_type = genomic DNA
attattctgagaaaagg

SEQ ID NO: 5 - DNA, 17 bp, Naturally occurring sequence
  source 1..17: mol_type = genomic DNA
tactttcttagaaaatt

SEQ ID NO: 6 - DNA, 17 bp, Naturally occurring sequence
  source 1..17: mol_type = genomic DNA
ggtgttcctagaagagg

SEQ ID NO: 7 - DNA, 27 bp, Naturally occurring sequence
  source 1..27: mol_type = genomic DNA
agcttagctatgactcatccggaagct

SEQ ID NO: 8 - DNA, 24 bp, Naturally occurring sequence
  source 1..24: mol_type = genomic DNA
gtattagtcatcgctattaccatg

SEQ ID NO: 9 - DNA, 24 bp, Naturally occurring sequence
  source 1..24: mol_type = genomic DNA
gatagcggtttgactcacggggat

SEQ ID NO: 10 - DNA, 61 bp, synthetic construct
  source 1..61: mol_type = other DNA
agggttcctggaagggaattattctgagaaaaggagcttagctatgactcatccggaagct

SEQ ID NO: 11 - DNA, 58 bp, synthetic construct
  source 1..58: mol_type = other DNA
cagattccgggaatccctactttcttagaaaattgtattagtcatcgctattaccatg

SEQ ID NO: 12 - DNA, 58 bp, synthetic construct
  source 1..58: mol_type = other DNA
atccttctgggaattctggtgttcctagaagagggatagcggtttgactcacggggat

SEQ ID NO: 13 - DNA, 177 bp, synthetic construct
  source 1..177: mol_type = other DNA
agggttcctggaagggaattattctgagaaaaggagcttagctatgactcatccggaagctcagattccgggaatccctactttcttagaaaattgtattagtcatcgctattaccatgatccttctgggaattctggtgttcctagaagagggatagcggtttgactcacggggat

SEQ ID NO: 14 - DNA, 31 bp, Naturally occurring sequence
  source 1..31: mol_type = genomic DNA
agagggtatataatggaagctcgacttccag

SEQ ID NO: 15 - DNA, 1656 bp, Naturally occurring sequence
  source 1..1656: mol_type = genomic DNA
atggaagatgccaaaaacattaagaaaggcccagcgccattctacccactcgaagacgggaccgctggcgagcagctgcataaagccatgaagcgctacgccctggtgcccggcaccatcgcctttaccgacgcacatatcgaggtggacattacctacgccgagtacttcgagatgagcgttcggctggcagaagctatgaagcgctatgggctgaatacaaaccatcggatcgtggtgtgtagcgagaatagcttgcagttcttcatgcccgtgttgggtgccctgttcatcggtgtggctgtggccccagctaacgacatctacaacgagcgcgagctgctgaacagcatgggcatcagccagcccaccgtcgtattcgtgagcaagaaagggctgcaaaagatcctcaacgtgcaaaagaagctaccgatcatacaaaagatcatcatcatggatagcaagaccgactaccagggcttccaaagcatgtacaccttcgtgacttcccatttgccacccggcttcaacgagtacgacttcgtgcccgagagcttcgaccgggacaaaaccatcgccctgatcatgaacagtagtggcagtaccggattgcccaagggcgtagccctaccgcaccgcaccgcttgtgtccgattcagtcatgcccgcgaccccatcttcggcaaccagatcatccccgacaccgctatcctgagcgtggtgccatttcaccacggcttcggcatgttcaccacgctgggctacttgatctgcggctttcgggtcgtgctcatgtaccgcttcgaggaagagctattcttgcgcagcttgcaagactataagattcaatctgccctgctggtgcccacactatttagcttcttcgctaagagcactctcatcgacaagtacgacctaagcaacttgcacgagatcgccagcggcggggcgccgctcagcaaggaggtaggtgaggccgtggccaaacgcttccacctaccaggcatccgccagggctacggcctgacagaaacaaccagcgccattctgatcacccccgaaggggacgacaagcctggcgcagtaggcaaggtggtgcccttcttcgaggctaaggtggtggacttggacaccggtaagacactgggtgtgaaccagcgcggcgagctgtgcgtccgtggccccatgatcatgagcggctacgttaacaaccccgaggctacaaacgctctcatcgacaaggacggctggctgcatagcggcgacatcgcctactgggacgaggacgagcacttcttcatcgtggaccggctgaagagcctgatcaaatacaagggctaccaggtagccccagccgaactggagagcatcctgctgcaacaccccaacatcttcgacgccggggtcgccggcctgcccgacgacgatgccggcgagctgcccgccgcagtcgtcgtgctggaacacggtaaaaccatgaccgagaaggagatcgtggactatgtggccagccaggttacaaccgccaagaagctgcgcggtggtgttgtgttcgtggacgaggtgcctaaaggactgaccggcaagttggacgcccgcaagatccgcgagattctcattaaggccaagaagggcggcaagatcgccgtctgataa

SEQ ID NO: 16 - DNA, 1951 bp, synthetic construct
  source 1..1951: mol_type = other DNA
agggttcctggaagggaattattctgagaaaaggagcttagctatgactcatccggaagctcagattccgggaatccctactttcttagaaaattgtattagtcatcgctattaccatgatccttctgggaattctggtgttcctagaagagggatagcggtttgactcacggggatgatatcaagatctagactctagagggtatataatggaagctcgacttccagcttggcattccggtactgttggtaaaaagcttggcaatccggtactgttggtaaactcgaggccaccatggaagatgccaaaaacattaagaaaggcccagcgccattctacccactcgaagacgggaccgctggcgagcagctgcataaagccatgaagcgctacgccctggtgcccggcaccatcgcctttaccgacgcacatatcgaggtggacattacctacgccgagtacttcgagatgagcgttcggctggcagaagctatgaagcgctatgggctgaatacaaaccatcggatcgtggtgtgtagcgagaatagcttgcagttcttcatgcccgtgttgggtgccctgttcatcggtgtggctgtggccccagctaacgacatctacaacgagcgcgagctgctgaacagcatgggcatcagccagcccaccgtcgtattcgtgagcaagaaagggctgcaaaagatcctcaacgtgcaaaagaagctaccgatcatacaaaagatcatcatcatggatagcaagaccgactaccagggcttccaaagcatgtacaccttcgtgacttcccatttgccacccggcttcaacgagtacgacttcgtgcccgagagcttcgaccgggacaaaaccatcgccctgatcatgaacagtagtggcagtaccggattgcccaagggcgtagccctaccgcaccgcaccgcttgtgtccgattcagtcatgcccgcgaccccatcttcggcaaccagatcatccccgacaccgctatcctgagcgtggtgccatttcaccacggcttcggcatgttcaccacgctgggctacttgatctgcggctttcgggtcgtgctcatgtaccgcttcgaggaagagctattcttgcgcagcttgcaagactataagattcaatctgccctgctggtgcccacactatttagcttcttcgctaagagcactctcatcgacaagtacgacctaagcaacttgcacgagatcgccagcggcggggcgccgctcagcaaggaggtaggtgaggccgtggccaaacgcttccacctaccaggcatccgccagggctacggcctgacagaaacaaccagcgccattctgatcacccccgaaggggacgacaagcctggcgcagtaggcaaggtggtgcccttcttcgaggctaaggtggtggacttggacaccggtaagacactgggtgtgaaccagcgcggcgagctgtgcgtccgtggccccatgatcatgagcggctacgttaacaaccccgaggctacaaacgctctcatcgacaaggacggctggctgcatagcggcgacatcgcctactgggacgaggacgagcacttcttcatcgtggaccggctgaagagcctgatcaaatacaagggctaccaggtagccccagccgaactggagagcatcctgctgcaacaccccaacatcttcgacgccggggtcgccggcctgcccgacgacgatgccggcgagctgcccgccgcagtcgtcgtgctggaacacggtaaaaccatgaccgagaaggagatcgtggactatgtggccagccaggttacaaccgccaagaagctgcgcggtggtgttgtgttcgtggacgaggtgcctaaaggactgaccggcaagttggacgcccgcaagatccgcgagattctcattaaggccaagaagggcggcaagatcgccgtctgataa